European Patent Application EP 4 527 397 A1, published March 26, 2025. Title: THERAPEUTIC USE OF A POSTBIOTIC COMPOSITION IN DYSLIPIDEMIAS. Applicant: IGEN BIOLAB GROUP AG. Application EP. The sequence listing filed with the application follows.

SEQUENCE LISTING (10 sequences)

SEQ ID NO: 1 - DNA, 20 bp, Danio rerio
  source 1..20: mol_type = other DNA
  primer_bind 1..20
gaacgacccacccatggagg

SEQ ID NO: 2 - DNA, 20 bp, Danio rerio
  source 1..20: mol_type = other DNA
  primer_bind 1..20
tgatgacctgagcgttgaag

SEQ ID NO: 3 - DNA, 20 bp, Danio rerio
  source 1..20: mol_type = other DNA
  primer_bind 1..20
catccacatggctctgagtg

SEQ ID NO: 4 - DNA, 20 bp, Danio rerio
  source 1..20: mol_type = other DNA
  primer_bind 1..20
ctcatccacaaagaagcggt

SEQ ID NO: 5 - DNA, 20 bp, Danio rerio
  source 1..20: mol_type = other DNA
  primer_bind 1..20
gagaaagcttgccaaacagg

SEQ ID NO: 6 - DNA, 20 bp, Danio rerio
  source 1..20: mol_type = other DNA
  primer_bind 1..20
gagggtcttgcaggagacag

SEQ ID NO: 7 - DNA, 20 bp, Danio rerio
  source 1..20: mol_type = other DNA
  primer_bind 1..20
ctgaggctctggtggacgtg

SEQ ID NO: 8 - DNA, 18 bp, Danio rerio
  source 1..18: mol_type = other DNA
  primer_bind 1..18
gcagctacgatgttggcg

SEQ ID NO: 9 - DNA, 20 bp, Danio rerio
  source 1..20: mol_type = other DNA
  primer_bind 1..20
cgtcgtcaggtgtttacggt

SEQ ID NO: 10 - DNA, 20 bp, Danio rerio
  source 1..20: mol_type = other DNA
  primer_bind 1..20
aggcacttctggaatcgaca